European Patent Application EP 4 242 237 A1, published September 13, 2023. Title: FokI NUCLEASE DOMAIN MUTANT. Applicant: EditForce, Inc. KYUSHU UNIVERSITY, NATIONAL UNIVERSITY CORPORATION. The sequence listing filed with the application follows.

SEQUENCE LISTING (20 sequences)

SEQ ID NO: 1 - protein, 579 aa, Flavobacterium okeanokoites
MVSKIRTFGWVQNPGKFENLKRVVQVFDRNSKVHNEVKNIKIPTLVKESKIQKELVAIMNQHDLIYTYKELVGTGTSIRSEAPCDAIIQATIADQGNKKGYIDNWSSDGFLRWAHALGFIEYINKSDSFVITDVGLAYSKSADGSAIEKEILIEAISSYPPAIRILTLLEDGQHLTKFDLGKNLGFSGESGFTSLPEGILLDTLANAMPKDKGEIRNNWEGSSDKYARMIGGWLDKLGLVKQGKKEFIIPTLGKPDNKEFISHAFKITGEGLKVLRRAKGSTKFTRVPKRVYWEMLATNLTDKEYVRTRRALILEILIKAGSLKIEQIQDNLKKLGFDEVIETIENDIKGLINTGIFIEIKGRFYQLKDHILQFVIPNRGVTKQLVKSELEEKKSELRHKLKYVPHEYIELIEIARNSTQDRILEMKVMEFFMKVYGYRGKHLGGSRKPDGAIYTVGSPIDYGVIVDTKAYSGGYNLPIGQADEMQRYVEENQTRNKHINPNEWWKVYPSSVTEFKFLFVSGHFKGNYKAQLTRLNHITNCNGAVLSVEELLIGGEMIKAGTLTLEEVRRKFNNGEINF

SEQ ID NO: 2 - protein, 196 aa, Flavobacterium okeanokoites
QLVKSELEEKKSELRHKLKYVPHEYIELIEIARNSTQDRILEMKVMEFFMKVYGYRGKHLGGSRKPDGAIYTVGSPIDYGVIVDTKAYSGGYNLPIGQADEMQRYVEENQTRNKHINPNEWWKVYPSSVTEFKFLFVSGHFKGNYKAQLTRLNHITNCNGAVLSVEELLIGGEMIKAGTLTLEEVRRKFNNGEINF

SEQ ID NO: 3 - DNA, 17 bp, Artificial Sequence
  Target Sequence of TALEN-A
agccgaaatcatcgcag

SEQ ID NO: 4 - DNA, 15 bp, Artificial Sequence
  Target Sequence of GFP_TALEN(L)
cagcgtgtccggcga

SEQ ID NO: 5 - DNA, 15 bp, Artificial Sequence
  Target Sequence of GFP_TALEN(R)
ttgccgtaggtggca

SEQ ID NO: 6 - DNA, 14 bp, Artificial Sequence
  Target Sequence of B2M_TALEN(L)
ccaaagattcaggt

SEQ ID NO: 7 - DNA, 14 bp, Artificial Sequence
  Target Sequence of B2M_TALEN(R)
gactttccattctc

SEQ ID NO: 8 - DNA, 50 bp, Artificial Sequence
  Target Site of TALEN-A
agccgaaatcatcgcagccgctgccgcgagctcctgcgatgatttcggct

SEQ ID NO: 9 - DNA, 42 bp, Artificial Sequence
  Target Site of GFP_TALEN
cagcgtgtccggcgagggcgagggcgatgccacctacggcaa

SEQ ID NO: 10 - DNA, 47 bp, Artificial Sequence
  Target Site of B2M_TALEN
ccaaagattcaggtttactcacgtcatccagcagagaatggaaagtc

SEQ ID NO: 11 - protein, 196 aa, Artificial Sequence
  M47 mutant
QLMKSELEEKKSELRRKLKYVPHEYIELIEIARNSTQYRIFEMKVMEFLVKVYGYRGKHLGGSRNPDGAIYTVGSPIDYGVIIDTKAYSGGYNLPIGQADAMLRYVEENQTRNKHINPNEWWKVYPSSVTEFKFLFVSGHFKGNYKAQLTRLNHITNCNGAVLSVEELLIGGEMIKAGTLTLEEVRRKFNNGEINF

SEQ ID NO: 12 - protein, 196 aa, Artificial Sequence
  M48 mutant
QLVKSELEEKKSELRHKLKYVPHEYIELIEIARNPTLDRILEMKVMEFFMKVYGYRGKHLGGSRKPDGVIYTVGSPIDYGVIVDTKAYSRGYNLPIGQADEMHRYVVENQTRNKLINPNEWWKVYPSSVTEFKFLFVSGHFKGNYKAQLTRLNHITNCKGAVLSVEELLIGGEMIRAGTLTLEEVRSKFNNGEINF

SEQ ID NO: 13 - protein, 196 aa, Artificial Sequence
  M49 mutant
QLMKSELEEKKFELRRKLKYVPHEYIELIEIARNSTQYRIFEMKVMEFLVKVYGYRGKHLGGSRNPDGAIYTVGSPIDYGVIVDTKAYSGGYNLPIGQADAMLRYVEENQTRNKHINPNEWWKVYPSSVTEFKFLFVSGHFKGNYKAQLTRLNHITNCNGAVLSVEELLIGGEMIKAGTLTLEEVRRKFNNGEINF

SEQ ID NO: 14 - protein, 196 aa, Artificial Sequence
  M50 mutant
QPVKSELEEKKAELRHKLKYVPHEYIELIEIARNSTQDRILEMMVMEFFMKVYGYRGKHLGGSRKPDGVIYTVGSPFDYGVIVDTKAYSRGYNLPIGHADEMQRYVQENQTRNKHINPNEWWKVYPSSVTEFKFLFVSGHFKGNYKAQLTRLNHITNCTGAVLSVEELLIGGEMIRAGTLTLEEVRSKFNNGEINF

SEQ ID NO: 15 - DNA, 14 bp, Artificial Sequence
  Target Sequence of B2M_PPR(L)
aatggaaagtcaaa

SEQ ID NO: 16 - DNA, 14 bp, Artificial Sequence
  Target Sequence of B2M_PPR(R)
agcaattcaggaaa

SEQ ID NO: 17 - DNA, 15 bp, Artificial Sequence
  Target Sequence of GFP_PPR(L)
acgacttcttcaagt

SEQ ID NO: 18 - DNA, 15 bp, Artificial Sequence
  Target Sequence of GFP_PPR(R)
cctggacgtagcctt

SEQ ID NO: 19 - DNA, 96 bp, Artificial Sequence
  Target Site of B2M_PPR
tactccaaagattcaggtttactcacgtcatccagcagagaatggaaagtcaaatttcctgaattgctatgtgtctgggtttcatccatccgacat

SEQ ID NO: 20 - DNA, 212 bp, Artificial Sequence
  Target Site of GFP_PPR
caagttcagcgtgtccggcgagggcgagggcgatgccacctacggcaagctgaccctgaagttcatctgcaccaccggcaagctgcccgtgccctggcccaccctcgtgaccaccctgacctacggcgtgcagtgcttcagccgctaccccgaccacatgaagcagcacgacttcttcaagtccgccatgcccgaaggctacgtccaggagc